European Patent Specification EP 3 809 838 B1, published April 1, 2026. Title: GENETICALLY MODIFIED MOUSE MODELS OF ALZHEIMER DISEASE. Applicant: THE JACKSON LABORATORY INDIANA UNIVERSITY RESEARCH AND TECHNOLOGY CORPORATION SAGE BIONETWORKS. Application Not Yet Assigned. The sequence listing filed with the application follows.

SEQUENCE LISTING (50 sequences)

SEQ ID NO: 1 - protein, 317 aa, Homo sapiens [sequence omitted]

SEQ ID NO: 2 - DNA, 2792 bp, Homo sapiens
actggccaatcacaggcaggaagatgaaggttctgtgggctgcgttgctggtcacattcctggcaggtatgggggcggggcttgctcggttccccccgctcctccccctctcatcctcacctcaacctcctggccccattcaggcagaccctgggccccctcttctgaggcttctgtgctgcttcctggctctgaacagcgatttgacgctctctgggcctcggtttcccccatccttgagataggagttagaagttgttttgttgttgttgtttgttgttgttgttttgtttttttgagatgaagtctcgctctgtcgcccaggctggagtgcagtggcgggatctcggctcactgcaagctccgcctcccaggtccacgccattctcctgcctcagcctcccaagtagctgggactacaggcacatgccaccacacccgactaacttttttgtattttcagtagagacggggtttcaccatgttggccaggctggtctggaactcctgacctcaggtgatctgcccgtttcgatctcccaaagtgctgggattacaggcgtgagccaccgcacctggctgggagttagaggtttctaatgcattgcaggcagatagtgaataccagacacggggcagctgtgatctttattctccatcacccccacacagccctgcctggggcacacaaggacactcaatacatgcttttccgctgggcgcggtggctcacccctgtaatcccagcactttgggaggccaaggtgggaggatcacttgagcccaggagttcaacaccagcctgggcaacatagtgagaccctgtctctactaaaaatacaaaaattagccaggcatggtgccacacacctgtgctctcagctactcaggaggctgaggcaggaggatcgcttgagcccagaaggtcaaggttgcagtgaaccatgttcaggccgctgcactccagcctgggtgacagagcaagaccctgtttataaatacataatgctttccaagtgattaaaccgactcccccctcaccctgcccaccatggctccaaagaagcatttgtggagcaccttctgtgtgcccctaggtactagatgcctggacggggtcagaaggaccctgacccaccttgaacttgttccacacaggatgccaggccaaggtggagcaagcggtggagacagagccggagcccgagctgcgccagcagaccgagtggcagagcggccagcgctgggaactggcactgggtcgcttttgggattacctgcgctgggtgcagacactgtctgagcaggtgcaggaggagctgctcagctcccaggtcacccaggaactgaggtgagtgtccccatcctggcccttgaccctcctggtgggcggctatacctccccaggtccaggtttcattctgcccctgtcgctaagtcttggggggcctgggtctctgctggttctagcttcctcttcccatttctgactcctggctttagctctctggatatctctctctcagctttgtctctctctcttcccttctgactcagtctctcacactcgtcctggctctgtctctgtccttccctagctcttttatatagagacagagagatggggtctcactgtgttgcccaggctggtcttgaacttctgggctcaagcgatcctcccgcctcggcctcccaaagtgctgggattagaggcatgagccaccttgcccggcctcctagctccttcttcgtctctgcctctgccctctgcatctgctctctgcatctgtctctgtctccttctctcggcctctgccccgttccttctctccctcttgggtctctctggctcatccccatctcgcccgccccatcccagcccttctccccgcctcccactgtgcgacaccctcccgccctctcggccgcagggcgctgatggacgagaccatgaaggagttgaaggcctacaaatcggaactggaggaacaactgaccccggtggcggaggagacgcgggcacggctgtccaaggagctgcaggcggcgcaggcccggctgggcgcggacatggaggacgtgcgcggccgcctggtgcagtaccgcggcgaggtgcaggccatgctcggccagagcaccgaggagctgcgggtgcgcctcgcctcccacctgcgcaagctgcgtaagcggctcctccgcgatgccgatgacctgcagaagcgcctggcagtgtaccaggccggggcccgcgagggcgccgagcgcggcctcagcgccatccgcgagcgcctggggcccctggtggaacagggccgcgtgcgggccgccactgtgggctccctggccggccagccgctacaggagcgggcccaggcctggggcgagcggctgcgcgcgcggatggaggagatgggcagccggacccgcgaccgcctggacgaggtgaaggagcaggtggcggaggtgcgcgccaagctggaggagcaggcccagcagatacgcctgcaggccgaggccttccaggcccgcctcaagagctggttcgagcccctggtggaagacatgcagcgccagtgggccgggctggtggagaaggtgcaggctgccgtgggcaccagcgccgcccctgtgcccagcgacaatcactgaacgccgaagcctgcagccatgcgaccccacgccaccccgtgcctcctgcctccgcgcagcctgcagcgggagaccctgtccccgccccagccgtcctcctggggtggaccctagtttaataaagattcaccaagtttcacgca

SEQ ID NO: 3 - protein, 249 aa, Artificial Sequence
  Synthetic Polypeptide
MGPLHQFLLLLITALSQALNTTVLQGMAGQSLRVSCTYDALKHWGRHKAWCRQLGEEGPCQRVVSTHGVWLLAFLKKRNGSTVIADDTLAGTVTITLKNLQAGDAGLYQCQSLRGREAEVLQKVLVEVLEDPLDDQDAGDLWVPEESSSFEGAQVEHSTSRQVSSCGSPLAYHLPPLSKESRDLLPTHLHSSPPGLRSPEQVSCSQHPLGCGQGQAEAGNTCGQRAGLWPRCWAPTSDPHWTRRYVREF

SEQ ID NO: 4 - DNA, 1056 bp, Artificial Sequence
  Synthetic Polynucleotide
acttcaagggaaaagcaagatcttgcacaaggtcccctccggctggctgctggcaaaggaaaggtgccatgggacctctccaccagtttctcctgctgctgatcacagccctgtcccaagccctcaacaccacggtgctgcagggcatggccggccagtccttgagggtgtcatgtacttatgacgccttgaagcactgggggagacacaaagcatggtgtcggcagctgggtgaggagggcccatgccagcgtgtggtgagcacacacggtgtgtggctgctggccttcctgaagaagcggaatgggagcacagtcatcgcagatgacacccttgctggaaccgtcaccatcactctgaagaacctccaagccggtgacgcgggcctctaccagtgtcagagtctccgaggccgagaggctgaggtcctgcagaaagtactggtggaggtgctggaggaccctctagatgaccaagatgctggagatctctgggtccccgaggagtcatcgagtttcgagggtgcccaagtggaacacagcacctccaggcaggtttcatcctgtgggtcacctctagcctaccaccttcctcctctttccaaggaatcaagagacctccttcccacccacctccattcttctcctcctggcctgcgttctcctgagcaagtttcttgcagccagcatcctctgggctgtggccaggggcaggcagaagccgggaacacctgtggtcagagggctggactgtggccaagatgctgggcaccaacttcagatcctcactggacccggaggtacgtgagagaattctgagtgggaggagaactacagcttaagtccagccaggagtcaatccagcctgcatgctctcccctcctccaccaagacttctgtttctgctacttttgcttcagaggccgcctctgcctcaagcccacctatcctgggagcaggaatactggtgtgtacatctgtgttgagtggggaagacagctggatggttgtctgtcaacttctgcactttggacattaaacattctccacacaccaa

SEQ ID NO: 5 - protein, 249 aa, Mus musculus
MGPLHQFLLLLITALSQALNTTVLQGMAGQSLRVSCTYDALKHWGRRKAWCRQLGEEGPCQRVVSTHGVWLLAFLKKRNGSTVIADDTLAGTVTITLKNLQAGDAGLYQCQSLRGREAEVLQKVLVEVLEDPLDDQDAGDLWVPEESSSFEGAQVEHSTSRQVSSCGSPLAYHLPPLSKESRDLLPTHLHSSPPGLRSPEQVSCSQHPLGCGQGQAEAGNTCGQRAGLWPRCWAPTSDPHWTRRYVREF

SEQ ID NO: 6 - DNA, 1056 bp, Mus musculus
acttcaagggaaaagcaagatcttgcacaaggtcccctccggctggctgctggcaaaggaaaggtgccatgggacctctccaccagtttctcctgctgctgatcacagccctgtcccaagccctcaacaccacggtgctgcagggcatggccggccagtccttgagggtgtcatgtacttatgacgccttgaagcactgggggagacgcaaggcctggtgtcggcagctgggtgaggagggcccatgccagcgtgtggtgagcacacacggtgtgtggctgctggccttcctgaagaagcggaatgggagcacagtcatcgcagatgacacccttgctggaaccgtcaccatcactctgaagaacctccaagccggtgacgcgggcctctaccagtgtcagagtctccgaggccgagaggctgaggtcctgcagaaagtactggtggaggtgctggaggaccctctagatgaccaagatgctggagatctctgggtccccgaggagtcatcgagtttcgagggtgcccaagtggaacacagcacctccaggcaggtttcatcctgtgggtcacctctagcctaccaccttcctcctctttccaaggaatcaagagacctccttcccacccacctccattcttctcctcctggcctgcgttctcctgagcaagtttcttgcagccagcatcctctgggctgtggccaggggcaggcagaagccgggaacacctgtggtcagagggctggactgtggccaagatgctgggcaccaacttcagatcctcactggacccggaggtacgtgagagaattctgagtgggaggagaactacagcttaagtccagccaggagtcaatccagcctgcatgctctcccctcctccaccaagacttctgtttctgctacttttgcttcagaggccgcctctgcctcaagcccacctatcctgggagcaggaatactggtgtgtacatctgtgttgagtggggaagacagctggatggttgtctgtcaacttctgcactttggacattaaacattctccacacaccaa

SEQ ID NO: 7 - DNA, 20 bp, Artificial Sequence
  Synthetic Polynucleotide
gaagcactgggggagacgca

SEQ ID NO: 8 - DNA, 183 bp, Artificial Sequence
  Synthetic Polynucleotide
gccctcaacaccacggtgctgcagggcatggccggccagtccttgagggtgtcatgtacttatgacgccttgaagcactgggggagacacaaagcatggtgtcggcagctgggtgaggagggcccatgccagcgtgtggtgagcacacacggtgtgtggctgctggccttcctgaagaagcgg

SEQ ID NO: 9 - DNA, 4980 bp, Mus musculus
cctgtatctcagggttgagagggaagagagtggggtttccagatgcccacatcccttgatacctagtcctcacccaactctgctctcctagtgaacaactggttggctacagtaacgctgggccaggcaggcatgcatgcgacgtattaccacaaagccagtgaccaggtgagccggagggagcgcctagctgtgggtcccaggctgggtttgctggtgcagttggtatgcccaggagtcctaatgggccactcacatgtgtgccgggccctctctcccccagctgcaggtgggtgtggagtttgaggccagcaccaggatgcaggacaccagtgcctcctttgggtatcagctggacctgcccaaggccaacttcctttttaaaggtaaggaaggcctcagcttccctcctggggaacaggccagataagactcagctgtctgtggtagagtccatgggaaatagggaggttgaacatgtgctggtggagtgggcggggactctgtgcagctccaaattactctgggtggcttgtcaaacagtggggctcctaccctggcatgtttagtacatgttgggggcctcgctttaagccctctcttcccattcccatctagcaagctctctggccctccccactcactcttaccttacttggagttcttctattgtgtgatgaaacactatgatggtaaacagcttagggagcaaagaggttatgttgggttacaactctcaggtggcatgcctaccactgaggagaagatggggcaggactcagcagaaagctgaaggcaagctgatgcagaaggccttgtgggagtgctgcttgttggcttgctccttatggcttcctcagcctgctcttatagcctccggaccattagcccagggtgccccactgaaaataatctgggtactcccacatcaatcacttagaaagtgccctacaggcttgcctgctgccctagctaatggagacatatgtattgaggttccctcagctggatctcttgagttcaagaccagcctggtctacagagcaagttctgggacagccagggctacccagagaaaccctgtctcagaaaagaaaaaaaagaaaaaggtgggggtggggtgactagcttgtataaaactagccagcacagcagggaagctgtgtgaatagtgacagccaggttcagaacctcattctgcgcagtgacatgggtttgtcaagcctgggcggtgttgagccacttaaagggttgctgtgatggtctggagtggccttggttgtgacttaggacatacgggtccgttgtggctaccatagagatgggtggccaggcacatcaagccacccagtctctgccccgctctcggcccacaggctctgtgaacagtaactggatcgtgggcgccacgctggagaagaagcttccgcccttgcccctgacactgtccctctgcgccttcctgaaccaccgcaagaataagttcctgtgtggcttcggcctcaccatcggctgagccctcctgtccttcctctgcagaccatcgctgggccggctgccctcccctcctctccctctctcttggggttggggcagtgggaaggaggggacctcccatgcccaaggatccccagcgccaggggacagtgcccagggggcctggggtcccggagggagtcctgggatctgaagggcattcgattgtgagcgcccaggcagaggcgcagaggcggctgtacacaggctcagaaaggaaagacttgatgtcctcctgagggcagcagaggagcgccgagccgcctgtcacttccccctccacccctccatagaaatcatgtttataagttatggaaaaccgggacattttacagaaaaaaaaaaacttaaaaaacaaaaaatatacgtggaaaaaaaaataggatctgggaggcctcggttttctccagttgttgacatggttgccagcaggcggcgccgagggttcagaaagcacagcagcaccaagcagtttagagaaagcttggccaggcatggtcacaccctctgctcttggggacttacactgccggaacatcagaggcctggcctcaccaggagggtggctccaggtcactcgcctctgtgcagtctggccccgagagctggcagaggactttgtctctgtaaacagggtgggggcagggagacggggctcaggagcctccctgtcccaaaacgggctgaggtggtagcttgtgctgactttctcccagtgggaaggtcagaggtctcagaaacttcaggaagaaacggagttcctggaagttcagcacaataaggaaagttactctgggaggaacgggccctagcaccttcccaggctgaaacaggaaatgtcaagttgttttgttttttaaattttgttgaagatgtagctctgggcctcacgtgtcaggcaggtgctgctgggttccctatagtgcttttccgtgaggcctgctctggggtgtgcgataagggcctcagattgggctctgcatctcactgctgcacctcatggcatcccaagggaagcaaagactcacgatgaactggtcagtgtcctagaccgcagcactaagaccctctctactgcctgggctggagatgggagctggcccttagcaacccatgaaaatcatctcaccacacccagtccttgccagtgttttctgaagccaaagctaacaggcctgggcctggccaggcaccctgtacgtacccttggagccaggtgttccgcctctgcccatcctgcagaatcatgttttgccgtgtctggtgccaaacactgctatgtggcttctctcctgccatcaacagctgggaacagggaaccttgtgcaggcagtgcttctagcaagcttgctgtggtctctgagccccttgtcctacctgacttcccaggtacaatggctttcccactttttgggggttttgttgttgttgggtttttttttgtttttcaagacagggtttctctgtgtagtcctgtcggtcctggaactcactttgtagaccaggctggcctccaactcagaaattcacctgcctctgcctccaagtgctgggattatgggattaaaggcatgtgccaccacgcccagctggcttttccactttttagccaggacttcattctattacctgagctcgggatcttcctgcctcagctttgcatatggctagcactatagacccatgttccagtgaatgacttatggcttgtctttttttttttttttttttttttttatgtgcattagtgttttgcctgcatgtatgccttcgtgagggtagcagatcttggtgttacagttgtgagctgctgtgtgggtgctgcgattttgaacctaggtcctgtgaaatgcagtcagtgctcctaacctctgagtcatctctccagctcctgctcttctgcttttatgaggaaaaagaaaagagaagtggcttgagagtggaaaatgcacatgcaggggtgcacacctgcagtcccagcatgctacagcagaggcagaaggacctttgtgggttagagggcagcctgagaatcttatctcaaaacaactttttaaaatgtgctctgtaggggtagctcttccctcccaaggtgacacatctggcaatcgccagaaacagatcaggagcatcaacgcttggtttcccagggcttggcttaatgtatggcttcaaacccatcgggagccaccactgaacagctcctgaaggaactggagcacgtcccagccttggaatggaaagagttcacctgtggtggaggaatcaacaacgagggatcccagaacaacgatcttcaccccagaagctgagcctcttagcccccacccacccatttccatttaggctgccagctcttttctttacaatgcaccagaccccgcggggaaagggaaggagcggttctcagtgccccagtaccaaggcctggattattcaatgaggtgtccgctccctttgttggcgggggaggggagcggggggtcacaaggcatccaaactccacctctttcctctgccctgctgtgaagggggagagaacaacccgcctcgtgacagggggctggcacagcccgccctagccctgaggagggggcgggacagggggagtcctataattggaccggtctgggatccgatcccctgctcagaccctggaggctaaggacttgtttcggaaggagctggtaagacaagctgggctggggattcacccagggaccttggtaggatgtgggctgggaaccttgagatcccccggagtccaggaaacaggcacaagaattggaaaagcaggcagcacgatagaagtcttgggggacaaactaaggactcgaggtaactagcctttgccagagtcagagcaggtggaggggttacctccaggaaggagtacgggactgtcggtgcacggcgtaccggctcaactaggaaccatcctatggcgaaaaaactcgggatgagccttaggctgcttttatataaatacctactgatttccatcacagtccccaagtaacccggactggtttcaaactgtggctcctcatggctgagctccctaagttctgtagttgtgggagggtaccacttcgcagggatggaggacgattaaaaatcgtgttaaattaacacaaaatggaaagcaggacttagccgggaagaaagaggaatgtaagctggaccacccgctggccctctgtgaagtggaatttgaaccctaggagagggagctggaatttttggcagcggatccaccccggggtgccgagatagcgaactcggcaaggggaggtaaacagacctttgggaagagcgggtgctctgttttggagatgtttgtgatggctcacagatctgagaagggaagatggggttctctgggtggccggagtccctccacccccgccccctggtgttcaaagacaatttttccctccgcag

SEQ ID NO: 10 - DNA, 4292 bp, Homo sapiens
actggccaatcacaggcaggaagatgaaggttctgtgggctgcgttgctggtcacattcctggcaggtatgggggcggggcttgctcggttccccccgctcctccccctctcatcctcacctcaacctcctggccccattcaggcagaccctgggccccctcttctgaggcttctgtgctgcttcctggctctgaacagcgatttgacgctctctgggcctcggtttcccccatccttgagataggagttagaagttgttttgttgttgttgtttgttgttgttgttttgtttttttgagatgaagtctcgctctgtcgcccaggctggagtgcagtggcgggatctcggctcactgcaagctccgcctcccaggtccacgccattctcctgcctcagcctcccaagtagctgggactacaggcacatgccaccacacccgactaacttttttgtattttcagtagagacggggtttcaccatgttggccaggctggtctggaactcctgacctcaggtgatctgcccgtttcgatctcccaaagtgctgggattacaggcgtgagccaccgcacctggctgggagttagaggtttctaatgcattgcaggcagatagtgaataccagacacggggcagctgtgatctttattctccatcacccccacacagccctgcctggggcacacaaggacactcaatacatgcttttccgctgggcgcggtggctcacccctgtaatcccagcactttgggaggccaaggtgggaggatcacttgagcccaggagttcaacaccagcctgggcaacatagtgagaccctgtctctactaaaaatacaaaaattagccaggcatggtgccacacacctgtgctctcagctactcaggaggctgaggcaggaggatcgcttgagcccagaaggtcaaggttgcagtgaaccatgttcaggccgctgcactccagcctgggtgacagagcaagaccctgtttataaatacataatgctttccaagtgattaaaccgactcccccctcaccctgcccaccatggctccaaagaagcatttgtggagcaccttctgtgtgcccctaggtactagatgcctggacggggtcagaaggaccctgacccaccttgaacttgttccacacaggatgccaggccaaggtggagcaagcggtggagacagagccggagcccgagctgcgccagcagaccgagtggcagagcggccagcgctgggaactggcactgggtcgcttttgggattacctgcgctgggtgcagacactgtctgagcaggtgcaggaggagctgctcagctcccaggtcacccaggaactgaggtgagtgtccccatcctggcccttgaccctcctggtgggcggctatacctccccaggtccaggtttcattctgcccctgtcgctaagtcttggggggcctgggtctctgctggttctagcttcctcttcccatttctgactcctggctttagctctctggatatctctctctcagctttgtctctctctcttcccttctgactcagtctctcacactcgtcctggctctgtctctgtccttccctagctcttttatatagagacagagagatggggtctcactgtgttgcccaggctggtcttgaacttctgggctcaagcgatcctcccgcctcggcctcccaaagtgctgggattagaggcatgagccaccttgcccggcctcctagctccttcttcgtctctgcctctgccctctgcatctgctctctgcatctgtctctgtctccttctctcggcctctgccccgttccttctctccctcttgggtctctctggctcatccccatctcgcccgccccatcccagcccttctccccgcctcccactgtgcgacaccctcccgccctctcggccgcagggcgctgatggacgagaccatgaaggagttgaaggcctacaaatcggaactggaggaacaactgaccccggtggcggaggagacgcgggcacggctgtccaaggagctgcaggcggcgcaggcccggctgggcgcggacatggaggacgtgcgcggccgcctggtgcagtaccgcggcgaggtgcaggccatgctcggccagagcaccgaggagctgcgggtgcgcctcgcctcccacctgcgcaagctgcgtaagcggctcctccgcgatgccgatgacctgcagaagcgcctggcagtgtaccaggccggggcccgcgagggcgccgagcgcggcctcagcgccatccgcgagcgcctggggcccctggtggaacagggccgcgtgcgggccgccactgtgggctccctggccggccagccgctacaggagcgggcccaggcctggggcgagcggctgcgcgcgcggatggaggagatgggcagccggacccgcgaccgcctggacgaggtgaaggagcaggtggcggaggtgcgcgccaagctggaggagcaggcccagcagatacgcctgcaggccgaggccttccaggcccgcctcaagagctggttcgagcccctggtggaagacatgcagcgccagtgggccgggctggtggagaaggtgcaggctgccgtgggcaccagcgccgcccctgtgcccagcgacaatcactgaacgccgaagcctgcagccatgcgaccccacgccaccccgtgcctcctgcctccgcgcagcctgcagcgggagaccctgtccccgccccagccgtcctcctggggtggaccctagtttaataaagattcaccaagtttcacgcatctgctggcctccccctgtgatttcctctaagccccagcctcagtttctctttctgcccacatactggccacacaattctcagccccctcctctccatctgtgtctgtgtgtatctttctctctgcccttttttttttttttagacggagtctggctctgtcacccaggctagagtgcagtggcacgatcttggctcactgcaacctctgcctcttgggttcaagcgattctgctgcctcagtagctgggattacaggctcacaccaccacacccggctaatttttgtatttttagtagagacgagctttcaccatgttggccaggcaggtctcaaactcctgaccaagtgatccacccgccggcctcccaaagtgctgagattacaggcctgagccaccatgcccggcctctgcccctctttcttttttagggggcagggaaaggtctcaccctgtcacccgccatcacagctcactgcagcctccacctcctggactcaagtgataagtgatcctcccgcctcagcctttccagtagctgagactacaggcgcataccactaggattaatttgggggggggggtggtgtgtgtggagatggggtctggctttgttggccaggctgatgtggaattcctgggctcaagcgatactcccaccttggcctcctgagtagctgagactactggctagcaccaccacacccagctttttattattatttgtagagacaaggtctcaatatgttgcccaggctagtctcaaacccctgggctcaagagatcctccgccatcggcctcccaaagtgctgggattccaggcatggggctccgagcccggcctgcccaacttaataatacttgttcctcagagttgcaactccaaatgacctgagattggtgcctttattctaagctattttcattttttttctgctgtcattattctcccccttctctcctccagtcttatctgatatctgcctccttcccacccaccctgcaccccatcccacccctctgtctctccctgttctcctcaggagactctggcttcctgttttcctccacttctatcttttatctctccctcctacggtttcttttctttctccccggcctgcttgtttctcccccaacccccttcatctggatttcttcttctgccattcagtttggtttgagctctctgcttctccggttccctctgagctagctgtcccttcacccactgtgaactgggtttccctgcccaaccctcattctctttctttctttctttttttttttttttttttttttttttttttgagacagagtcttgctctgttgcccagcctggagtgcagtggtgcaatcttggttcactgcaacctccacttcccagattcaagcaattctcctgcctcagcctccagagtagctgggattacaggcgtgtcccaccacacccgactaatttttgtatttttggtagagacaaggcttcggcattgtt

SEQ ID NO: 11 - DNA, 1834 bp, Artificial Sequence
  Synthetic Polynucleotide
gaagttcctattctctagaaagtataggaacttcaggtctgaagaggagtttacgtccagccaagctagcttggctgcaggtcgtcgaaattctaccgggtaggggaggcgcttttcccaaggcagtctggagcatgcgctttagcagccccgctgggcacttggcgctacacaagtggcctctggcctcgcacacattccacatccaccggtaggcgccaaccggctccgttctttggtggccccttcgcgccaccttctactcctcccctagtcaggaagttcccccccgccccgcagctcgcgtcgtgcaggacgtgacaaatggaagtagcacgtctcactagtctcgtgcagatggacagcaccgctgagcaatggaagcgggtaggcctttggggcagcggccaatagcagctttgctccttcgctttctgggctcagaggctgggaaggggtgggtccgggggcgggctcaggggcgggctcaggggcggggcgggcgcccgaaggtcctccggaggcccggcattctgcacgcttcaaaagcgcacgtctgccgcgctgttctcctcttcctcatctccgggcctttcgacctgcagcctgttgacaattaatcatcggcatagtatatcggcatagtataatacgacaaggtgaggaactaaaccatgggatcggccattgaacaagatggattgcacgcaggttctccggccgcttgggtggagaggctattcggctatgactgggcacaacagacaatcggctgctctgatgccgccgtgttccggctgtcagcgcaggggcgcccggttctttttgtcaagaccgacctgtccggtgccctgaatgaactgcaggacgaggcagcgcggctatcgtggctggccacgacgggcgttccttgcgcagctgtgctcgacgttgtcactgaagcgggaagggactggctgctattgggcgaagtgccggggcaggatctcctgtcatctcaccttgctcctgccgagaaagtatccatcatggctgatgcaatgcggcggctgcatacgcttgatccggctacctgcccattcgaccaccaagcgaaacatcgcatcgagcgagcacgtactcggatggaagccggtcttgtcgatcaggatgatctggacgaagagcatcaggggctcgcgccagccgaactgttcgccaggctcaaggcgcgcatgcccgacggcgatgatctcgtcgtgacccatggcgatgcctgcttgccgaatatcatggtggaaaatggccgcttttctggattcatcgactgtggccggctgggtgtggcggaccgctatcaggacatagcgttggctacccgtgatattgctgaagagcttggcggcgaatgggctgaccgcttcctcgtgctttacggtatcgccgctcccgattcgcagcgcatcgccttctatcgccttcttgacgagttcttctgaggggatcaattctctagagctcgctgatcagcctcgactgtgccttctagttgccagccatctgttgtttgcccctcccccgtgccttccttgaccctggaaggtgccactcccactgtcctttcctaataaaatgaggaaattgcatcgcattgtctgagtaggtgtcattctattctggggggtggggtggggcaggacagcaagggggaggattgggaagacaatagcaggcatgctggggatgcggtgggctctatggcttctgaggcggaaagaaccagctggggctcgactagagcttgcggaacccttcgaagttcctattctctagaaagtataggaacttccatatg

SEQ ID NO: 12 - DNA, 5166 bp, Mus musculus
aaacctgatggagaagatacaggcctctgtggctaccaaccccatcatcaccccagtggcccaggagaatcaatgagtatccttctcctgtcctgcaacaacatccatatccagccaggtggccctgtctcaagcacctctctggccctctggtggcccttgcttaataaagattctccgagcacattctgagtctctgtgagtgattccaatcagcttcagcctcagtttattgttttttgccttacctagcacacattccatggccctgtcactatctgtagagggaggtggttttgcagcaatagaaatgaagcctaggacctagcaacataaaagaacaagtgatctaccactgagccacgcccacagcccctcactgggggattctaggcaggggctctaccactgagccacccgcagcccctcactggggaatcatatctaccactgagtcacgcccctccagcccctcactacgggaattctagtcagtagctctaccactgagccacacccacagcctctggggctcttcaccgccccctacccctggattctaggcatgggctcattttatttatttatttatttaagatttgtttatcttatgtataaggtacactgcagctgtcttcaggcgtcaggtcccattacagatggttgtgagccaccatgtggttgctgggaattgaactcaggacttatagaagagtagtcagtgctcttaactgctgagccatctctccagcacccagtacaggctcttctatttagctatatccacccttctttttagtctgaaataggatctcaactgattttccttgcactccctctagcctagtttggtcttgaatatttgaatctttgttttcaaatcaatctctacaggaactgagaaaggcatgtaccacttcatgtgggtcagttgggctacttttcccaacttcccaagcacccactgcacagctatgccttgaatcaatcaacatgtaagagaccagggtcgccaggcggtgtttacttttctggttgtcttatctctcctcctccgctctagtcttatctgacaccctctccttgccttgtctctcctctttttcccttctaggcttccttttctggcttcctgttttcctgatcctctgttatctcaccctcccgcggtttcttttgctctgggcctttggttggcggtttctacggtttctacgtggcttttggaacctcagcctttctcccttgctctgaagttagctggatctttgctccctctgggtcatggggccttagccccattctttctcccctgcctgtgctgcatgccttttgactttcccagcaagtgtatggagagtgagttcaggctggggacacaaaaccattctccccatgtcctggtactcaaaggggtcatggtggaagctggagagcccctggctggcttctcctcccaccccctcagttctcagggactcagcagggctcccactaacaggggcaggctagggcttgagctgtgtcttgggtcgggccaaggcttcagaactcaactgcctctggcacaccccgagcctgcagcttttcctggcatcaaactcagcattatctggaggcaggcaccactcccacacatgactcattaggcccaatgagaagatgggtcggtgggctagtgacagggccctagacagccacacttcatgcccaggggctaggagcacacccccagagcctcactactctcaaatatcaagatgaggggagagtatagagggaatgtctccctctgaagacctgaattattgtgatgttatttgagccacgctggccttgaactctgaaccctcctgcctcatcttcaaaggctggaattacaggttcgcgccactaggcctatctgagaacttagttaattctacagaagagagtttgttttcactggtttgaaacgaggcctcgtgtacccagagctactcttttgccaactcactgtagagccaaggatgaccttgaactctggtcttcctggctccgagtcctcggtactgggtagacaatgtgtgatcctaacccccagttttatgtggtgctatacagatggcatccagggtttcctgcatgctggacaggtcatcaaccaaccgagccacatcctcctcatcatcatcactttgttgttggttttcaatccagagctcatggagcccaagctggcctcaatctatataaccaagactgtgcctggtcttcctgtctctacctaacaaatgatggtgggatgcagggatgtacaaccaggagcagagccttacttctaaacgaagaaggaaccccacctccctgtgggcagacctggaggtggggcaaggaccacagaaagacattacagaactaggatcgtgaaggaagtcatggaggccagcctgttgtacagagtgagttccaggacagccagggctacacagaggaaaacaagaaggaaaaaaaaaaaaaaaaaaagaactgaatgactagcagttttagaaccttagctgtgtgcttcccgtaccctacctgtggcacaggaagcccttgttgctaagagtaggatgacactggaagcaccaagcactgggcagagtaagggggaaatctgttacattattcagatgggcgcttgaggactgagcaggactcctttcaagaagcaaaagggtcaggcctggtgcccacagggactggaagctagctagcgccgagttggccccagagatgtcgcaacccagccagggtcgagaatctgttccacccctttcacaaccatccccctgttgtcgtcgtccccacccccacccccgccccaactgacacgtgggttgcaggggcaccaggccagccaacctagagtctgggccccttagccaccagctgccagggggtcactgtcggtcaatgacagctctgggggagggggggagaagggccttggactctagcctgagagaaaggatgttgtggaaggagggggcagggaggcaagtttagggcctgcaggggcctaggaggccccacaagacctaaaaacgggggaaggggggttgtgccagttaggggacactatggagctctgcaagctaagaggctcttagcttctttgcagttttgactagctgaagaggcaacttctaaggaagggagatgaggggatgccaagatcccagagagcatccgaggaggtctgagggtgtgcagatgcaaaggcattggaggtgaagggagccagggtgcagcatccgggacagaatgtgagctgaggctcctggtcaaggagaaggtagagaagagctaacctgaggatgcagtgtgagctaggggtgagatgggggtgaggggagttgtttgtaagacccccccccttaaggtgggacagcctcagagagagagtgagtaggcagagcagccaaggctgggtggagatcaatgagatttggaagtgaggatgctgaccagtgacgagccttgggcctaaataaaaagcctggatgtgggatctgcctcccagtatcgaccagaatgacagaagagagtgggctggttgtgttggtgttggtgcatgcctgtaatcccagcaactcactagagaggcagaggcaggagcatcacaaattccaggccagccaaaaagcctatgtaaaaaaaaaaaaaagagaaaaaagaaaaaagaaaaagtaggtggacacagagacaagggggaggctcagggggagggcgaccagcttgctccgccccctccccaaccggttaaacctctgtgcaggatcctcccaccgccatgggcctcctgagagatccttagatccaggttagtgcataggaaagtgtccccccactacctacagctaagggattggggtggtgggatcatggtggagggcggtggtgaatactagcgatgtcccccgctacccgtgcgtctgcctccagggtgcccctccaaccaggatgaggctcttcatcgctcttcctgtcctgattgtggtcgtagccatgaccttggaaggtaagaaagagccttggaaggtaagaaagaggcttggaagtgtgaagttggccttgtgcctgcggcccaggcttagaagaccctcgaggagggctctgaggtccctttctgtgtcatcattccactaccgccctcccatcgtcccccatcccacctgccaggtgccttatttttgtgtcaaagtgggtgctgaaggaggcaactctgtccagaaaagacgcagtaaccaatgacctaggataccaccctttggaattggctaatcttcctagaaggggcggagcgtaaaaacaaggaggtgagaggtgcagtaaaatcaagtgtccaataccctcccccatgctaatgagtttgctcgcaaccctctcgcggcaggcccagcccccgcccaggcggccccggatttgtccggaacattggagagcataccggataaactgaaggagtttgggaacactttggaagacaaggcccgggcagccattgaacatatcaaacagaaggaaattttgaccaagacccggttaggacctttcagggcacgggcgggtggtgtgtgtgtgtgtgcgtgcgcgcgcgcccgtgtgtaaaagccctagcagacagttccacactgacacaatggggaaactgcaccagagtgtttgacactttccctgaagtcatagaactgtatctgaagtcattgaactggatgtcaaagtgctcgtagtgtggagacaggcggtgtaactcccagccaactgttagagatgtttccaagtcctagtgaagggccaagctaggcggctgactggttaggacagaccctgacccctccctgtgtactcttgagacaggtcatgacttgagtctccgagacagagaaagaatgtaggagagttggggcaggggcacagcagaagctgtacaggcctgggctctgcagtttacactggccaaagagagattagggcatgctgggttaagaactagccaggcagtggtggcgcacacctttgatcccagtattcatgaggcagaggcaggcagatctctttgaggccagcctgattggagctagttctaggaaagccagggctacacagagaaaccctgtctcaacaccaccaccacccccc

SEQ ID NO: 13 - protein, 311 aa, Mus musculus
MKALWAVLLVTLLTGCLAEGEPEVTDQLEWQSNQPWEQALNRFWDYLRWVQTLSDQVQEELQSSQVTQELTALMEDTMTEVKAYKKELEEQLGPVAEETRARLGKEVQAAQARLGADMEDLRNRLGQYRNEVHTMLGQSTEEIRARLSTHLRKMRKRLMRDAEDLQKRLAVYKAGAREGAERGVSAIRERLGPLVEQGRQRTANLGAGAAQPLRDRAQAFGDRIRGRLEEVGNQARDRLEEVREHMEEVRSKMEEQTQQIRLQAEIFQARLKGWFEPIVEDMHRQWANLMEKIQASVATNPIITPVAQENQ

SEQ ID NO: 14 - protein, 317 aa, Homo sapiens [sequence omitted]

SEQ ID NO: 15 - protein, 299 aa, Homo sapiens
KVEQAVETEPEPELRQQTEWQSGQRWELALGRFWDYLRWVQTLSEQVQEELLSSQVTQELRALMDETMKELKAYKSELEEQLTPVAEETRARLSKELQAAQARLGADMEDVRGRLVQYRGEVQAMLGQSTEELRVRLASHLRKLRKRLLRDADDLQKRLAVYQAGAREGAERGLSAIRERLGPLVEQGRVRAATVGSLAGQPLQERAQAWGERLRARMEEMGSRTRDRLDEVKEQVAEVRAKLEEQAQQIRLQAEAFQARLKSWFEPLVEDMQRQWAGLVEKVQAAVGTSAAPVPSDNH

SEQ ID NO: 16 - protein, 7 aa, Artificial Sequence
  Synthetic Polypeptide
PKKKRKV

SEQ ID NO: 17 - protein, 14 aa, Artificial Sequence
  Synthetic Polypeptide
RPAATKKAGQAKKK

SEQ ID NO: 18 - DNA, 6607 bp, Artificial Sequence
  Synthetic Polynucleotide
atggccttaggcacacagctgatgcttctgctgtggaaaaattacacctatcgacggagacaaccgatccaactactagtggagttgctttggcccctcttcctcttcttcatcctagtggctgtccgtcactcccacccccctctggagcatcacgaatgccactttccaaacaagccattaccatcggcgggcacggtgccctggctgcagggccttgtctgcaacgtaaacaactcctgcttccagcacccaacgcctggcgagaagcctggggtcctgagtaactttaaggattccttgatctcgaggctcctcgctgatacccgcacagtgctcgggggccacagcatccaggacatgctggatgccctggggaaactgatccccgtgctcagggcagttggaggtggagcacgaccacaggagagtgaccagccgaccagtcaagggtcagtgactaagcttctggagaagatcctgcaaagggcatccctggatcctgtgctgggtcaagcccaggattctatgagaaagttctcagatgctatcagggatcttgcccaggagctcctgacactgcccagcctgatggagctccgagctttgctgcggaggccccgagggtcagctggttctctggagctggtttcggaggccctctgcagtaccaagggacccagcagtccagggggcctgtccctcaattggtacgaagccaaccagcttaatgagttcatggggccagaggtggcccctgccctgcctgacaacagtctcagccctgcctgctctgagtttgtggggacactggatgaccaccctgtgtctcggctgctctggaggcgcctgaagccattgatcctcgggaaaattctctttgcacctgacacaaacttcactcggaagctcatggctcaggtgaaccagaccttcgaggagctggctctgttgagggacctacacgaactctggggggtgctgggaccccagatcttcaacttcatgaatgacagtaccaacgtggccatgcttcagaggcttctggatgtggggggcacagggcagaggcagcagacacccagagcccagaagaagttggaggctatcaaagactttctggatcctagtaggggtggctacagctggcgggaggcccacgcagatatgggacgcctggctggaatcctaggacaaatgatggagtgtgtgtccctggacaagctggaggctgtgccctcagaggaagctcttgtgtcccgtgccctggagctgctgggtgagcgccgcctctgggcaggcatcgtgttcctgagcccagagcatcctctggacccatccgaactgtcatctccagccctgagtcctggccacctacgattcaagattcgaatggatatcgatgatgtcacaaggaccaataagatcagggacaagttttgggacccaggtccgtcagcagatcctttcatggaccttcggtatgtgtggggaggcttcgtgtacctgcaggacctgctggagcaggcagctgtgcgagtgctcggtggcgggaactcccgcacaggtctctacctgcagcagatgccacacccctgctacgtggatgatgtgttcctgcgggtgctgagccggtctctgcctctgtttctgactctggcctggatttattcggtggcgctcactgtgaaggccgtggtgcgtgagaaagagacacggctgcgagaaaccatgcgtgcgatggggctgagccgcgcggtgctctggcttggttggttcctcagctgcctgggacccttcctggtcagcgctgcgttgctggtattagtgcttaagctagggaacatccttccttacagccacccggttgtaatcttccttttcttggcggccttcgcggtggccaccgtcgctcagagttttctgctcagcgccttcttctccagggccaacctggcagcagcctgcggggggctcgcctattttgcgctctatctgccctacgtactgtgtgtggcctggcgcgagcgcctgcacctgggcggactcttagctgcgagcctgctgtcccctgtagcctttggctttggatgcgaaagcctggcgctactagaggagcagggagacggggctcagtggcacaatttgggcacaggccccgcggaggacgtcttcagcctggcccaggtgtctgccttcctgttgcttgatgccgtcatctacggccttgccctctggtacctagaggctgtgtgcccaggccagtatggaatccctgaaccatggaatttcccttttcggaggagctactggtgtggacctgggcctcccaagagttctgtcttggcccctgccccacaagatcccaaggttctggtggaagagccaccccttggcctggttcctggtgtctccattcgaggcctgaagaaacattttcgtggctgtccgcagccagccctgcaaggactcaaccttgacttctacgaaggccacatcactgcctttttgggtcacaacggggctggcaagacaaccacactgtccattttgagtggtctcttcccacccagtagtggctcggcctccatcctgggccatgatgtacaaaccaacatggcagccatccggccccacctgggcatctgcccgcagtacaatgtgctgtttgatatgctgacagtggaagaacatgtttggttctatggccgtttgaaaggcgtgagtgcagccgccatgggccccgagcgggaacgtctgatacgggatgtggggcttaccctcaagcgggacacacagacacgccacctctctggtggaatgcagagaaaactttctgtggccattgcctttgtgggtggctctcgtgtggtcatcatggacgagcccactgctggtgtggaccccgcttcccgccgtggcatttgggaattgctacttaagtacagagaaggtcggacactgattctctccactcaccacctggatgaggcagagctcttgggagatcgcgtggccatggtggcaggtggctctttgtgctgctgtgggtccccgcttttcttgcgccgacacttgggctgcggttactacctgaccctggtgaagagttctcagtccctcgtcacccatgatgctaagggagacagtgaggaccccagacgggaaaagaagtcagatggcaatggcaggacgtcagacacagcgttcacacgaggaacctcagacaagagcaaccaggccccggctcctggcgccgttcccatcaccccaagcacagcccggatactagagctagtgcagcagcatgtgcctggagcacaactcgtggaggacctgccccatgagcttctgcttgtgctaccctatgcgggggccctggatggcagcttcgccatggtcttccaggagctggatcagcagctggagctcctgggtctcacaggctacgggatctcggacaccaacctggaggagatcttcctaaaggtggtggaggatgcgcacagagaaggtggggactctagaccgcagctgcaccttcgcacatgcactccacagccccccacagggccagaggcatcagttctggagaatggggagctggccccacagggcttggcacccaacgctgcccaagtgcaaggctggacacttacctgtcaacagctccgggctctgctccacaagcgttttctgcttgctcgccgcagccgccggggcctgtttgcacaggttgtgttgcctgccctctttgtgggcctggccctgttcttcagcctcattgtgcctccttttggccagtacccacccctgcagctcagccctgctatgtatggccctcaggtctcgttcttcagtgaggatgcccctggggaccccaaccggatgaagctgctggaggctctgctaggggaggctgggctgcaggaacccagtatgcaggacaaagatgccaggggatctgagtgtacacactccctagcttgctacttcacggtccctgaggtccctcctgatgtggccagcatcctggccagtggcaactggacgccagaatctccatccccagcttgccaatgcagtcagcctggagcccgccgcctgttgccagattgcccggctggagctgggggtccaccacccccccaggctgtggctggcttgggggaggtggtccagaacctcactggccgaaatgtgtctgactttttggtgaagacataccccagcctggtgcgccgaggcctaaagaccaagaagtgggtggatgaggtcagatatgggggcttctccctgggaggccgagatccagacctgcccacagggcatgaggtggtccgcacattggcagagattcgggcactgctgagcccccaacctgggaatgcgctagaccgtatcctgaacaacctcactcagtgggcccttggccttgatgctcggaacagcctcaagatctggttcaacaacaagggctggcatgccatggtggcctttgtgaaccgagccaacaatggactcctacatgccctcctaccatctggtccagtccgccatgcccacagcatcactacactcaaccatcctttgaacttgaccaaggagcagctatctgaagctacactgatagcctcctctgtggatgtccttgtctccatctgtgtggtcttcgccatgtcatttgtcccagccagctttaccctggtcctcatagaggaacgcatcaccagagccaagcatctgcagctggtcagcggcctgccccaaaccctctattggcttggcaacttcctctgggacatgtgtaactacttggtggcagtgtgcatagtggtgttcatcttcctagcctttcagcagagagcctatgtggccccagagaacctgcctgctctcttactcttgcttctgctgtatgggtggtctatcacaccactcatgtacccagcctccttcttcttctcagtgcccagcacggcctatgtggtgctcacctgcatcaacctcttcattggcatcaatagcagcatggccaccttcgtgctagaactgctttcagatcagaacctgcaagaagtgagccggatcctgaaacaagtgtttcttattttcccccacttttgccttggccgagggctcattgacatggttcggaaccaggccatggcagatgcctttgagcgcttaggagacaagcaatttcagtcacccctacgctgggacatcattggcaagaacctcctggccatgatggcccagggacctctgttcctcctcatcacactcctgctccaacaccgcaaccgtctcctgccacaatcaaaaccaagactgctgccgcccctgggggaggaggatgaggatgtggctcaagagcgtgagcgggtgaccaagggggctacccagggggatgtgctagtcctcagggacttgaccaaggtttaccgtgggcagaggaacccagctgtggatcgcctgtgcttagggatcccccctggggagtgtttcgggctgctgggtgtcaacggggcagggaagacatccaccttccgcatggtgacaggggacacactgcccagcagtggtgaagcagtactggcaggccacaacgtggcccaggagcggtctgccgcacaccgcagcatgggctactgtccccagtctgatgccatcttcgacctgctgaccggccgggaacatctggaactgtttgctcgcctgcgcggggtgcccgaggcccaagttgcccagactgcgctctctggcctggtgcgcctgggccttcctagctatgcagaccgacccgcgggtacctacagcggaggcaacaaacggaagctggcgacagccttagctctggttggtgacccagctgtggtctttctggacgagcccaccacaggcatggacccaagtgcgcggcgatttctttggaacagcttgctgtccgtggtgcgcgagggccgctccgtagtgctcacgtcgcacagcatggaggagtgcgaagcgctctgcacgcgcctggccatcatggtgaacgggcggttccgctgtctgggaagctctcagcatctcaaaggcaggttcggggctggccacacactgactctaagggtcccaccggaccagcctgagccggcgatagccttcatcaggatcacattccctggggctgaactccgggaggtgcacggcagccgtctgcgcttccaactgccaccggggggcagatgcaccctgacacgagtgttcagggagctggctgcccagggcagggcccacggtgtggaggacttctctgtgagccagaccactctggaggaggtgttcctatatttctccaaagaccaaggggaagaggaagagagcagtcggcaggaggctgaagaagaggaggtttccaaacctggccggcagcatcccaaacgtgtcagccgattcctggaagaccccagctctgtggagaccatgatctgagcatgcctgccttgggactgagtggcaaagctcagacagaggatctctgtaccatacgctggctcccagaaagccttgggctctgggggaaataaaaagaaactagaatgagaaaaaaaaaaaaaaa

SEQ ID NO: 19 - protein, 2167 aa, Artificial Sequence
  Synthetic Polypeptide
MALGTQLMLLLWKNYTYRRRQPIQLLVELLWPLFLFFILVAVRHSHPPLEHHECHFPNKPLPSAGTVPWLQGLVCNVNNSCFQHPTPGEKPGVLSNFKDSLISRLLADTRTVLGGHSIQDMLDALGKLIPVLRAVGGGVRPQESDQPTSQGSVTKLLEKILQRASLDPVLGQAQDSMRKFSDAIRDLAQELLTLPSLMELRALLRRPRGSAGSLELVSEALCSTKGPSSPGGLSLNWYEANQLNEFMGPEVAPALPDNSLSPACSEFVGTLDDHPVSRLLWRRLKPLILGKILFAPDTNFTRKLMAQVNQTFEELALLRDLHELWGVLGPQIFNFMNDSTNVAMLQRLLDVGGTGQRQQTPRAQKKLEAIKDFLDPSRGGYSWREAHADVGRLAGILGQMMECVSLDKLEAVPSEEALVSRALELLGERRLWAGIVFLSPEHPLDPSELSSPALSPGHLRFKIRMDIDDVTRTNKIRDKFWDPGPSADPFMDLRYVWGGFVYLQDLLEQAAVRVLGGGNSRTGLYLQQMPHPCYVDDVFLRVLSRSLPLFLTLAWIYSVALTVKAVVREKETRLRETMRAMGLSRAVLWLGWFLSCLGPFLVSAALLVLVLKLGNILPYSHPVVIFLFLAAFAVATVAQSFLLSAFFSRANLAAACGGLAYFALYLPYVLCVAWRERLHLGGLLAASLLSPVAFGFGCESLALLEEQGDGAQWHNLGTGPAEDVFSLAQVSAFLLLDAVIYGLALWYLEAVCPGQYGIPEPWNFPFRRSYWCGPGPPKSSVLAPAPQDPKVLVEEPPLGLVPGVSIRGLKKHFRGCPQPALQGLNLDFYEGHITAFLGHNGAGKTTTLSILSGLFPPSSGSASILGHDVQTNMAAIRPHLGICPQYNVLFDMLTVEEHVWFYGRLKGVSAAAMGPERERLIRDVGLTLKRDTQTRHLSGGMQRKLSVAIAFVGGSRVVIMDEPTAGVDPASRRGIWELLLKYREGRTLILSTHHLDEAELLGDRVAMVAGGSLCCCGSPLFLRRHLGCGYYLTLVKSSQSLVTHDAKGDSEDPRREKKSDGNGRTSDTAFTRGTSDKSNQAPAPGAVPITPSTARILELVQQHVPGAQLVEDLPHELLLVLPYAGALDGSFAMVFQELDQQLELLGLTGYGISDTNLEEIFLKVVEDAHREGGDSRPQLHLRTCTPQPPTGPEASVLENGELAKLVLDPQAPQGLAPNAAQVQGWTLTCQQLRALLHKRFLLARRSRRGLFAQVVLPALFVGLALFFSLIVPPFGQYPPLQLSPAMYGPQVSFFSEDAPGDPNRMKLLEALLGEAGLQEPSMQDKDARGSECTHSLACYFTVPEVPPDVASILASGNWTPESPSPACQCSQPGARRLLPDCPAGAGGPPPPQAVAGLGEVVQNLTGRNVSDFLVKTYPSLVRRGLKTKKWVDEVRYGGFSLGGRDPDLPTGHEVVRTLAEIRALLSPQPGNALDRILNNLTQWALGLDARNSLKIWFNNKGWHAMVAFVNRANNGLLHALLPSGPVRHAHSITTLNHPLNLTKEQLSEGTLIASSVDVLVSICVVFAMSFVPASFTLVLIEERITRAKHLQLVSGLPQTLYWLGNFLWDMCNYLVAVCIVVFIFLAFQQRAYVAPENLPALLLLLLLYGWSITPLMYPDSFFFSVPSTAYVVLTCINLFIGINSSMATFVLELLSDQNLQEVSRILKQVFLIFPHFCLGRGLIDMVRNQAMADAFERLGDKQFQSPLRWDIIGKNLLAMMAQGPLFLLITLLLQHRNRLLPQSKPRLLPPLGEEDEDVAQERERVTKGATQGDVLVLRDLTKVYRGQRNPAVDRLCLGIPPGECFGLLGVNGAGKTSTFRMVTGDTLPSSGEAVLAGHNVAQERSAAHRSMGYCPQSDAIFDLLTGREHLELFARLRGVPEAQVAQTALSGLVRLGLPSYADRPAGTYSGGNKRKLATALALVGDPAVVFLDEPTTGMDPSARRFLWNSLLSVVREGRSVVLTSHSMEECEALCTRLAIMVNGRFRCLGSSQHLKGRFGAGHTLTLRVPPDQPEPAIAFIRITFPGAELREVHGSRLRFQLPPGGRCTLTRVFRELAAQGRAHGVEDFSVSQTTLEEVFLYFSKDQGEEEESSRQEAEEEEVSKPGRQHPKRVSRFLEDPSSVETMI

SEQ ID NO: 20 - protein, 2167 aa, Mus musculus
MALGTQLMLLLWKNYTYRRRQPIQLLVELLWPLFLFFILVAVRHSHPPLEHHECHFPNKPLPSAGTVPWLQGLVCNVNNSCFQHPTPGEKPGVLSNFKDSLISRLLADTRTVLGGHSIQDMLDALGKLIPVLRAVGGGVRPQESDQPTSQGSVTKLLEKILQRASLDPVLGQAQDSMRKFSDAIRDLAQELLTLPSLMELRALLRRPRGSAGSLELVSEALCSTKGPSSPGGLSLNWYEANQLNEFMGPEVAPALPDNSLSPACSEFVGTLDDHPVSRLLWRRLKPLILGKILFAPDTNFTRKLMAQVNQTFEELALLRDLHELWGVLGPQIFNFMNDSTNVAMLQRLLDVGGTGQRQQTPRAQKKLEAIKDFLDPSRGGYSWREAHADVGRLAGILGQMMECVSLDKLEAVPSEEALVSRALELLGERRLWAGIVFLSPEHPLDPSELSSPALSPGHLRFKIRMDIDDVTRTNKIRDKFWDPGPSADPFMDLRYVWGGFVYLQDLLEQAAVRVLGGGNSRTGLYLQQMPHPCYVDDVFLRVLSRSLPLFLTLAWIYSVALTVKAVVREKETRLRETMRAMGLSRAVLWLGWFLSCLGPFLVSAALLVLVLKLGNILPYSHPVVIFLFLAAFAVATVAQSFLLSAFFSRANLAAACGGLAYFALYLPYVLCVAWRERLHLGGLLAASLLSPVAFGFGCESLALLEEQGDGAQWHNLGTGPAEDVFSLAQVSAFLLLDAVIYGLALWYLEAVCPGQYGIPEPWNFPFRRSYWCGPGPPKSSVLAPAPQDPKVLVEEPPLGLVPGVSIRGLKKHFRGCPQPALQGLNLDFYEGHITAFLGHNGAGKTTTLSILSGLFPPSSGSASILGHDVQTNMAAIRPHLGICPQYNVLFDMLTVEEHVWFYGRLKGVSAAAMGPERERLIRDVGLTLKRDTQTRHLSGGMQRKLSVAIAFVGGSRVVIMDEPTAGVDPASRRGIWELLLKYREGRTLILSTHHLDEAELLGDRVAMVAGGSLCCCGSPLFLRRHLGCGYYLTLVKSSQSLVTHDAKGDSEDPRREKKSDGNGRTSDTAFTRGTSDKSNQAPAPGAVPITPSTARILELVQQHVPGAQLVEDLPHELLLVLPYAGALDGSFAMVFQELDQQLELLGLTGYGISDTNLEEIFLKVVEDAHREGGDSRPQLHLRTCTPQPPTGPEASVLENGELAKLVLDPQAPQGLAPNAAQVQGWTLTCQQLRALLHKRFLLARRSRRGLFAQVVLPALFVGLALFFSLIVPPFGQYPPLQLSPAMYGPQVSFFSEDAPGDPNRMKLLEALLGEAGLQEPSMQDKDARGSECTHSLACYFTVPEVPPDVASILASGNWTPESPSPACQCSQPGARRLLPDCPAGAGGPPPPQAVAGLGEVVQNLTGRNVSDFLVKTYPSLVRRGLKTKKWVDEVRYGGFSLGGRDPDLPTGHEVVRTLAEIRALLSPQPGNALDRILNNLTQWALGLDARNSLKIWFNNKGWHAMVAFVNRANNGLLHALLPSGPVRHAHSITTLNHPLNLTKEQLSEATLIASSVDVLVSICVVFAMSFVPASFTLVLIEERITRAKHLQLVSGLPQTLYWLGNFLWDMCNYLVAVCIVVFIFLAFQQRAYVAPENLPALLLLLLLYGWSITPLMYPDSFFFSVPSTAYVVLTCINLFIGINSSMATFVLELLSDQNLQEVSRILKQVFLIFPHFCLGRGLIDMVRNQAMADAFERLGDKQFQSPLRWDIIGKNLLAMMAQGPLFLLITLLLQHRNRLLPQSKPRLLPPLGEEDEDVAQERERVTKGATQGDVLVLRDLTKVYRGQRNPAVDRLCLGIPPGECFGLLGVNGAGKTSTFRMVTGDTLPSSGEAVLAGHNVAQERSAAHRSMGYCPQSDAIFDLLTGREHLELFARLRGVPEAQVAQTALSGLVRLGLPSYADRPAGTYSGGNKRKLATALALVGDPAVVFLDEPTTGMDPSARRFLWNSLLSVVREGRSVVLTSHSMEECEALCTRLAIMVNGRFRCLGSSQHLKGRFGAGHTLTLRVPPDQPEPAIAFIRITFPGAELREVHGSRLRFQLPPGGRCTLTRVFRELAAQGRAHGVEDFSVSQTTLEEVFLYFSKDQGEEEESSRQEAEEEEVSKPGRQHPKRVSRFLEDPSSVETMI

SEQ ID NO: 21 - DNA, 126 bp, Mus musculus
gatgcagaattcggacatgattcaggatttgaagtccgccatcaaaaactggtgttctttgctgaagatgtgggttcgaacaaaggcgccatcatcggactcatggtgggcggcgttgtcatagca

SEQ ID NO: 22 - DNA, 126 bp, Artificial Sequence
  Synthetic Polynucleotide
gatgcagaattccgacatgattcaggatatgaagtccatcatcaaaaactggtgttctttgctgaagatgtgggttcgaacaaaggcgccatcatcggactcatggtgggcggcgttgtcatagca

SEQ ID NO: 23 - protein, 42 aa, Artificial Sequence [sequence omitted]

SEQ ID NO: 24 - DNA, 127 bp, Mus musculus
atgaccaccatggtcaacgtggacacccttccagaatatgagaagagtcagatcaagagagcgctggagttagggacggtgatgaccgtgttcaacgcccgcaaatccaccccagagcggaggacag

SEQ ID NO: 25 - protein, 50 aa, Mus musculus
MTTMVNVDTLPEYEKSQIKRALELGTVMTVFNARKSTPERRTVQMIMETR

SEQ ID NO: 26 - protein, 50 aa, Artificial Sequence
  Synthetic Polypeptide
MSTTVNVDSLAEYEKSQIKRALELGTVMTVFSFRKSTPERRTVQVIMETR

SEQ ID NO: 27 - DNA, 127 bp, Artificial Sequence
  Synthetic Polynucleotide
atgaccaccatggtcaacgtggacacccttccagaatatgagaagagtcagatcaagagagcgctggagttagggacggtgttgactgtgttcaacgcccgcaaatccaccccagagcggaggacag

SEQ ID NO: 28 - DNA, 127 bp, Artificial Sequence; identical to SEQ ID NO: 27
  Synthetic Polynucleotide

SEQ ID NO: 29 - protein, 50 aa, Artificial Sequence
  Synthetic Polypeptide
MTTMVNVDTLPEYEKSQIKRALELGTVLTVFNARKSTPERRTVQMIMETR

SEQ ID NO: 30 - DNA, 4113 bp, Artificial Sequence
  Synthetic Polynucleotide
atgaccaccatggtcaacgtggacacccttccagaatatgagaagagtcagatcaagagagcgctggagttagggacggtgttgaccgtgttcaacgcccgcaaatccaccccagagcggaggacagtacagatgatcatggagactcggcaggtggcatggagcaagaccgcagacaagattgaaggcttcctggacatcatggagataaaggaaatccgtccggggaagaactccaaggactttgagcgagccaaggctgtccgccacaaggcagaatgttgcttcaccatcctctacggcacccagtttgtcctcagcacgctcagtttggcaacggactcaaaggaggatgcggtgaagtggctctctggtttgaagatcctacaccaggaagcgatgagtgcatccacccccacaatgattgagagttggctgagaaaacagatttattcagtagatcaaacccgaagaaacagcatcagcctccgggagctgaagaccatcttgcccctggtcaacttcaaagtgagcggcatcaagtttctcaaggacaagctggtggaaatcggcgcacagaaagatgagctcagctttgaacagttccatctcttctataagaaactcatgtttgaccagcaaaaatcgatacttgacgaattcaaaaaagactcctccgtgttcatcctaggaaacacagaccggccggatgcctcggctgtctacctgcaggacttccaaaggtttcttttacatgaacagcaggagctatgggctcaggatctgaacaaagtccgggagcggatgaccaagtttatcgacgacacaatgagagagaccgcagagcccttcttatttgtggatgagttcctcacgtatctgttctcccgggagaacagcatctgggacgagaagtacgatgcagtggacatgcaggacatgaacaaccccttgtcccactactggatctcctcttcccacaacacgtacctcactggggaccagctgcgtagtgagtcctccacggaagcgtatatccgctgtctgcgcgctggttgccgctgcattgagctggactgctgggacgggcctgatgggaagcccattatctaccacggctggacacggaccaccaagatcaagtttgatgatgttgttcaggccatccgagaccacgcctttgttacctccagcttccccgtcatcttgtctatcgaggagcactgcagtgtggagcagcaacgtcacatggccaaggtgttcaaggaagtgttaggagacatgctgttgacgaagcccacagaggccagtgctgaccagctgccctcgcccagtcagcttcgtgagaagatcattatcaagcataagaagctgggtcccaagggtgatgtcgacgtcaacgtggaggacaagaaagatgagcacaagccccagggcgagctgtatatgtgggactccatcgaccagaaatggacgcgccactactgtgccattgctgacgccaagctgtccttcggtgatgacattgaacaggctgtggaggaggagccggtccaggacactccccccacggagctgcattttggggagaaatggttccacaagaaggtggagagtaggaccagtgcggagaagctgctgcaagagtactgtgctgagaccggggccaaggacggcaccttcctggtgcgggagagcgagaccttccccaatgactacacactctccttctggcggtctggccgggtgcagcactgccggatccggtctactatggagaatggggtcatgaagtactacctgaccgacaacctcacgttcaacagcatctacgccctcatccagcactaccgtgaggcacacctgcgctgcgcggagttcgagctgcggctcacagacccggtgcccaaccccaacccacacgagtccaagccgtggtactatgacagtctgagcaggggggaagcggaggacatgctgatgcggatcccccgagatggagccttcctcatccggaagagggaggggaccaactcctacgccatcaccttcagggccaggggcaaggtgaaacattgtcgcatcaaccgggacggacgccacttcgtgctgggcacctctgcctactttgagagcctggtggagcttgtcagctactacgagaagcacgcgctctatcgcaagatgaggcttcgataccccgtgaccccggagctcctggagcgatataatatggaaagagacatcaactctctttatgacgtcagcaggatgtatgtggacccaagtgagatcaacccttccatgcctcagaggaccgtgaaagcgctctatgactacaaagccaagcgcagcgacgagctgaccttctgccgcggtgccctcatccacaatgtctccaaggagcccgggggatggtggaaaggggactacgggacccggatccagcagtacttcccgtccaactatgtcgaggatatctcggcaggcgatgctgaggagatggaaaagcagattattgaagacaatcccctcgggtctctctgcaaaggcatattggatcttaatacctacaacgttgtgaaggccccccaggggaaaaaccagaaagccttcgtctttatcctggagcctaagaaacagggagatcctcccgtggagttcgcgaccgaccgtgtggaggagctgtttgagtggtttcagagcatacgggagatcacttggaagatggacaccaaggagaacaacatgaagtactgggagaggaaccagtccatcgccattgagctctcggacttggttgtatactgcaagccaactagcaaaaccaaggaccatttggaaaatcccgacttccgagaaatccgctcttttgtggagacgaaggcagacagcattgtcaggcaaaaacctgtcgatctattgcgatacaatcagaagggcctgacccgagtctaccccaagggacagagagttgactcttcgaactatgaccccttccgtctgtggctgtgcggctcccagatggtggcactcaatttccagactccagacaaatacatgcagatgaaccacgcgctgttttcgctcaatgggcgaacaggctacgtcctgcagcctgagagcatgcgctctgagaagtatgatccgatgcccctggagtcccagaggaagatcctgatgacactcactgtcaaggttcttggtgcacgccacctccctaaactagggcggagtattgcctgtccttttgtggaggtggaaatctgcggggctgagtatgacagcaacaaattcaagacgacggttgtgaatgacaatggcctcagccctgtctgggctccaactcaggagaaggtgacatttgagatctatgatccaaaccttgccttcctacgctttgtggtctacgaagaagacatgttcagtgatcccaacttcctggctcatgccacgtaccccattaaaggcatcaaatccgggtttagatcagtccctctgaagaatgggtacagtgaagacatcgagctggcatccctcctggttttctgtgagatgaggccagtcctggagagtgaagaggaactctattcctcctgtcgccaactgcggaggcggcaagaagagctcaacaaccagctcttcctttacgacacgcaccagaacctgcgcggagccaaccgtgatgccctggtgaaggagttcaatgttaacgagaatcagctgcagctgtaccaggagaagtgcaaccggaggctgagagagaagagagtaagcaacagcaggttctactcctagaagccgtgtgtgcgtgcgcgcatgcgcacggtgttcacgagcgcatctgggtacgggagagccttataaacagcccccaggaagagattcatctgtgacattcatcgtcctctctccgagccactcaccatagagatgacagttctgaagacgcccccgtgggcaggaggcgttgagaccttcctgctatttttccaccttggacaactttcttaacttatactacccctgatagaggatccccccaactgtgtgccttttgaacttccctgttctcagcctcattgaataaagacaacagtttcatgccgttaa

SEQ ID NO: 31 - protein, 1265 aa, Artificial Sequence
  Synthetic Polypeptide
MTTMVNVDTLPEYEKSQIKRALELGTVLTVFNARKSTPERRTVQMIMETRQVAWSKTADKIEGFLDIMEIKEIRPGKNSKDFERAKAVRHKAECCFTILYGTQFVLSTLSLATDSKEDAVKWLSGLKILHQEAMSASTPTMIESWLRKQIYSVDQTRRNSISLRELKTILPLVNFKVSGIKFLKDKLVEIGAQKDELSFEQFHLFYKKLMFDQQKSILDEFKKDSSVFILGNTDRPDASAVYLQDFQRFLLHEQQELWAQDLNKVRERMTKFIDDTMRETAEPFLFVDEFLTYLFSRENSIWDEKYDAVDMQDMNNPLSHYWISSSHNTYLTGDQLRSESSTEAYIRCLRAGCRCIELDCWDGPDGKPIIYHGWTRTTKIKFDDVVQAIRDHAFVTSSFPVILSIEEHCSVEQQRHMAKVFKEVLGDMLLTKPTEASADQLPSPSQLREKIIIKHKKLGPKGDVDVNVEDKKDEHKPQGELYMWDSIDQKWTRHYCAIADAKLSFGDDIEQAVEEEPVQDTPPTELHFGEKWFHKKVESRTSAEKLLQEYCAETGAKDGTFLVRESETFPNDYTLSFWRSGRVQHCRIRSTMENGVMKYYLTDNLTFNSIYALIQHYREAHLRCAEFELRLTDPVPNPNPHESKPWYYDSLSRGEAEDMLMRIPRDGAFLIRKREGTNSYAITFRARGKVKHCRINRDGRHFVLGTSAYFESLVELVSYYEKHALYRKMRLRYPVTPELLERYNMERDINSLYDVSRMYVDPSEINPSMPQRTVKALYDYKAKRSDELTFCRGALIHNVSKEPGGWWKGDYGTRIQQYFPSNYVEDISAGDAEEMEKQIIEDNPLGSLCKGILDLNTYNVVKAPQGKNQKAFVFILEPKKQGDPPVEFATDRVEELFEWFQSIREITWKMDTKENNMKYWERNQSIAIELSDLVVYCKPTSKTKDHLENPDFREIRSFVETKADSIVRQKPVDLLRYNQKGLTRVYPKGQRVDSSNYDPFRLWLCGSQMVALNFQTPDKYMQMNHALFSLNGRTGYVLQPESMRSEKYDPMPLESQRKILMTLTVKVLGARHLPKLGRSIACPFVEVEICGAEYDSNKFKTTVVNDNGLSPVWAPTQEKVTFEIYDPNLAFLRFVVYEEDMFSDPNFLAHATYPIKGIKSGFRSVPLKNGYSEDIELASLLVFCEMRPVLESEEELYSSCRQLRRRQEELNNQLFLYDTHQNLRGANRDALVKEFNVNENQLQLYQEKCNRRLREKRVSNSRFYS

SEQ ID NO: 32 - DNA, 26 bp, Artificial Sequence
  Synthetic Polynucleotide
acttgaccaaggagcagctatctgaa

SEQ ID NO: 33 - DNA, 27 bp, Artificial Sequence
  Synthetic Polynucleotide
gcagctatctgaagctacactgtgagt

SEQ ID NO: 34 - DNA, 149 bp, Artificial Sequence
  Synthetic Polynucleotide
aaaggttccaatccagtctccaccacccctgagcaacatgaccactgatagtaaatggatggactcacagtgtaccttcagatagctgctccttggtcaagttcaaaggatggttgagtgtagtgatctgtgggcatggcggactggac

SEQ ID NO: 35 - protein, 42 aa, Mus musculus
DAEFGHDSGFEVRHQKLVFFAEDVGSNKGAIIGLMVGGVVIA

SEQ ID NO: 36 - protein, 42 aa, Homo sapiens [sequence omitted]

SEQ ID NO: 37 - DNA, 21 bp, Artificial Sequence
  Synthetic Polynucleotide
tttgatggcggacttcaaatc

SEQ ID NO: 38 - DNA, 20 bp, Artificial Sequence
  Synthetic Polynucleotide
gtgaagatggatgcagaatt

SEQ ID NO: 39 - DNA, 127 bp, Artificial Sequence
  Synthetic Polynucleotide
ttcatctggccagacgcaatctcggggagaggcagtttatttttgcctaccagtttttgatgatggacttcatatcctgaatcatgtcggaattctgcatccatcttcacttccgagatctcttccg

SEQ ID NO: 40 - DNA, 20 bp, Artificial Sequence
  Synthetic Polynucleotide
gagagcgctggagttaggga

SEQ ID NO: 41 - DNA, 20 bp, Artificial Sequence
  Synthetic Polynucleotide
ggagctttgtctcctcccag

SEQ ID NO: 42 - DNA, 20 bp, Artificial Sequence
  Synthetic Polynucleotide
aaggagctttgtctcctccc

SEQ ID NO: 43 - DNA, 20 bp, Artificial Sequence
  Synthetic Polynucleotide
cctttaaaggcgacagctaa

SEQ ID NO: 44 - DNA, 20 bp, Artificial Sequence
  Synthetic Polynucleotide
gccgttttacacatagaact

SEQ ID NO: 45 - DNA, 20 bp, Artificial Sequence
  Synthetic Polynucleotide
ccttgctgctcggagtatgt

SEQ ID NO: 46 - DNA, 20 bp, Artificial Sequence
  Synthetic Polynucleotide
ctgaccccctcctctaaaga

SEQ ID NO: 47 - DNA, 702 bp, Artificial Sequence
  Synthetic Polynucleotide
tgtcagactcacaggctccacccccagcccacgtggatctgggaggtgccctcccctgggaggagacaaagctcctttaagaaaagcagggcagatatcagggcagcctggcttagcagtagtgttggagaagaagctagcaggcaggcagcagagacatggagctggcctcagcacatctccacaaagggcaggttccctggggaggactactgctcacaggtaaggagatattccttcccagtagagagcaggggagctcagagactggctgggctcttctgggagaggaaaggaacctgagaagggacatctggcttctgcttgaagcttgacggcaacaggaagctctcagtgagtgtgaattggctagtggtgaggagtaactcagttctttgctattgttaagtttatcgcactggctaggatatcctgaagactgaagtccacaactctgtcagggtgactctccacgtaaaaaccaaactggggcaagtaaacagaattattgcatactacactgagaaatttgcaaatacactaggctctgggacactgatttgcaaacaggtatatgagcatgttccaggcagcagggattaagccaaaacccacctagccctgcacacaaagccctagttctatgtgtaaaacggcagacctgcgagggcatctaggtggggtcaggttggcaagcacttc

SEQ ID NO: 48 - DNA, 503 bp, Mus musculus
caaatttgttgttggttctgacaataaagcttgggaatattctaaaacccttggaatggttcttagtctatagttatcacacattcacggtgattattattagaactcttcagggaagaagtaccctctcttactttttaaatttatgttgacaggatgggacttctgtggtatttgatgagtctgtccttctatgggatcctgcagagtcatgcttcgggtgagtatgtggtgctggataaatgactgaaattaatttaacatacaggatcctatatagtgaatttaaatgagcataatgttggttttgttccacagaattctgtagttgcatagaatcaagtgtctgaaagaaccatagaattaggggatgagagaaactagacaacttaggaaggggtctgatgagtataaacacagggacatctcttcaacttcatgccccacaggctaattctctgtattctcatctcaagtactgtggaggaaatggcagggagatt

SEQ ID NO: 49 - DNA, 2088 bp, Artificial Sequence
  Synthetic Polynucleotide
atgaaccatcaaaaagccaaggtcctcccagctgggcactgttatccatccctggggatgtgggcctcagaggctggctgcgtgaggctttctgtgccaccctctatcagcaggaatccagccatggtgaacgaggccagaggaagtggcagtcccaacccgcgatctgagggcagcagcagtggcagcgagagttccaaggacagttcaagatgttccacccccagcctggacccagagcggcacgagagactccgggagaagatgaggcgcagaatggactctggtgacaagtggttctccctggagttcttcccccctcgaactgctgagggagctgttaacctcatctccaggtttgaccggatggcagcagggggccccctcttcgtagatgttacctggcacccagctggagaccctggctcagacaaggagacctcctccatgatgatcgccagcacagcagtaaactactgcggcttggaaaccatcctgcatatgacctgctgccagcagcgcccggaggagatcacaggccatctgcacagagccaagcagctgggcctgaagaacataatggcgctgaggggagaccctgtaggtgaccactgggaagcagaggaaggaggcttcagctatgccacagacctggtgaagcacatccggaccgagtttgctgactattttgacatctgtgtggcaggttaccccagaggccaccccgatgcagagagcttcgaggatgacctgaagcatttgaaggagaaggtatctgcaggcgtcgacttcattatcactcagctcttctttgaggccagcaccttcttcagctttgtgaaggcctgcacagagataggcatctcttgccctatcctgcctgggatcttccctattcagggctacacttcccttcggcagcttgtaaaactgtccaagctggaggtgccacagaagatcaaggatgtaattgagcccatcaaagacaacgatgctgccatccgcaactacggcattgagctggctgtaagcctgtgccgggagctgctggacagtggcttggtgccaggcctccacttctataccctcaaccgcgaggtggccaccatggaggtgctaaagcaactgggcatgtggaccgaggaccccaggcgtcccttgccctgggctctcagtgcgcatcccaagcgccgggaggaagatgtccgtcccatcttctgggcctccagaccaaagagctacatctaccgcacacaggactgggatgagtttcctaacggccgctggggtaattcttcctcaccagcctttggggagctgaaagactactacctcttctacctgaaaagcaagtcccccagggaggagctgctgaagatgtggggcgaggagctcaccagcgaagagagtgtctttgaagtctttgaacactacctctctggagagccgaatcgccatggctacagagtaacctgcctgccctggaacgatgaacccctggcagcggaaaccagcctgatgaaggaagagctgctccgcgtgaacaggctgggcatcctcaccatcaactctcagcccaacatcaacgcaaaaccatcctcagaccctgttgtgggctggggccccagtgggggttatgtcttccagaaggcctacctcgaattcttcacctcccgtgaaactgtggaggcgcttctgcaggtgctgaagacatacgagctgcgggtcaactaccacatcgtggacgtgaagggagagaacatcactaatgcccctgagctgcagcccaatgccgtgacgtggggcatcttcccgggtcgagagatcatccagcctactgtggtggaccccatcagcttcatgttctggaaggatgaggcctttgccctgtggatcgagcagtggggcaagctatacgaggaggagtcgccatcccgcatgatcatccaatacatccatgacaactatttcctggtcaacctggtggacaacgagttcccgctggacagctgcctgtggcaggtggtggaggacacgtttgagctgctcaacaggcatcccacggagagagagacacaggctccatga

SEQ ID NO: 50 - protein, 695 aa, Artificial Sequence
  Synthetic Polypeptide
MNHQKAKVLPAGHCYPSLGMWASEAGCVRLSVPPSISRNPAMVNEARGSGSPNPRSEGSSSGSESSKDSSRCSTPSLDPERHERLREKMRRRMDSGDKWFSLEFFPPRTAEGAVNLISRFDRMAAGGPLFVDVTWHPAGDPGSDKETSSMMIASTAVNYCGLETILHMTCCQQRPEEITGHLHRAKQLGLKNIMALRGDPVGDHWEAEEGGFSYATDLVKHIRTEFADYFDICVAGYPRGHPDAESFEDDLKHLKEKVSAGVDFIITQLFFEASTFFSFVKACTEIGISCPILPGIFPIQGYTSLRQLVKLSKLEVPQKIKDVIEPIKDNDAAIRNYGIELAVSLCRELLDSGLVPGLHFYTLNREVATMEVLKQLGMWTEDPRRPLPWALSAHPKRREEDVRPIFWASRPKSYIYRTQDWDEFPNGRWGNSSSPAFGELKDYYLFYLKSKSPREELLKMWGEELTSEESVFEVFEHYLSGEPNRHGYRVTCLPWNDEPLAAETSLMKEELLRVNRLGILTINSQPNINAKPSSDPVVGWGPSGGYVFQKAYLEFFTSRETVEALLQVLKTYELRVNYHIVDVKGENITNAPELQPNAVTWGIFPGREIIQPTVVDPISFMFWKDEAFALWIEQWGKLYEEESPSRMIIQYIHDNYFLVNLVDNEFPLDSCLWQVVEDTFELLNRHPTERETQAP